European Patent Application EP 4 506 461 A1, published February 12, 2025. Title: 单碱基编辑修复HBA2基因突变的方法及其应用. Applicant: 广州瑞风生物科技有限公司. Application WO. The sequence listing filed with the application follows.

SEQUENCE LISTING (69 sequences)

SEQ ID NO: 1 - DNA, 20 bp, synthetic construct
  source 1..20: mol_type = other DNA
ccgtcaagctggagcctcgg

SEQ ID NO: 2 - DNA, 15 bp, synthetic construct
  source 1..15: mol_type = other DNA
aagctggagcctcgg

SEQ ID NO: 3 - DNA, 16 bp, synthetic construct
  source 1..16: mol_type = other DNA
caagctggagcctcgg

SEQ ID NO: 4 - DNA, 17 bp, synthetic construct
  source 1..17: mol_type = other DNA
tcaagctggagcctcgg

SEQ ID NO: 5 - DNA, 18 bp, synthetic construct
  source 1..18: mol_type = other DNA
gtcaagctggagcctcgg

SEQ ID NO: 6 - DNA, 19 bp, synthetic construct
  source 1..19: mol_type = other DNA
cgtcaagctggagcctcgg

SEQ ID NO: 7 - DNA, 21 bp, synthetic construct
  source 1..21: mol_type = other DNA
accgtcaagctggagcctcgg

SEQ ID NO: 8 - DNA, 22 bp, synthetic construct
  source 1..22: mol_type = other DNA
taccgtcaagctggagcctcgg

SEQ ID NO: 9 - DNA, 23 bp, synthetic construct
  source 1..23: mol_type = other DNA
ataccgtcaagctggagcctcgg

SEQ ID NO: 10 - DNA, 24 bp, synthetic construct
  source 1..24: mol_type = other DNA
aataccgtcaagctggagcctcgg

SEQ ID NO: 11 - DNA, 25 bp, synthetic construct
  source 1..25: mol_type = other DNA
aaataccgtcaagctggagcctcgg

SEQ ID NO: 12 - DNA, 19 bp, synthetic construct
  source 1..19: mol_type = other DNA
cgtcaagcaggagcctcgg

SEQ ID NO: 13 - DNA, 19 bp, synthetic construct
  source 1..19: mol_type = other DNA
tctcaagctggagcctcgg

SEQ ID NO: 14 - DNA, 19 bp, synthetic construct
  source 1..19: mol_type = other DNA
cgtcactgaggagcctcgg

SEQ ID NO: 15 - DNA, 20 bp, synthetic construct
  source 1..20: mol_type = other DNA
accgtcaagctggagcctcg

SEQ ID NO: 16 - DNA, 15 bp, synthetic construct
  source 1..15: mol_type = other DNA
caagctggagcctcg

SEQ ID NO: 17 - DNA, 16 bp, synthetic construct
  source 1..16: mol_type = other DNA
tcaagctggagcctcg

SEQ ID NO: 18 - DNA, 17 bp, synthetic construct
  source 1..17: mol_type = other DNA
gtcaagctggagcctcg

SEQ ID NO: 19 - DNA, 18 bp, synthetic construct
  source 1..18: mol_type = other DNA
cgtcaagctggagcctcg

SEQ ID NO: 20 - DNA, 19 bp, synthetic construct
  source 1..19: mol_type = other DNA
ccgtcaagctggagcctcg

SEQ ID NO: 21 - DNA, 21 bp, synthetic construct
  source 1..21: mol_type = other DNA
taccgtcaagctggagcctcg

SEQ ID NO: 22 - DNA, 22 bp, synthetic construct
  source 1..22: mol_type = other DNA
ataccgtcaagctggagcctcg

SEQ ID NO: 23 - DNA, 23 bp, synthetic construct
  source 1..23: mol_type = other DNA
aataccgtcaagctggagcctcg

SEQ ID NO: 24 - DNA, 24 bp, synthetic construct
  source 1..24: mol_type = other DNA
aaataccgtcaagctggagcctcg

SEQ ID NO: 25 - DNA, 25 bp, synthetic construct
  source 1..25: mol_type = other DNA
caaataccgtcaagctggagcctcg

SEQ ID NO: 26 - DNA, 20 bp, synthetic construct
  source 1..20: mol_type = other DNA
ataccgtcaagctggagcct

SEQ ID NO: 27 - DNA, 15 bp, synthetic construct
  source 1..15: mol_type = other DNA
gtcaagctggagcct

SEQ ID NO: 28 - DNA, 16 bp, synthetic construct
  source 1..16: mol_type = other DNA
cgtcaagctggagcct

SEQ ID NO: 29 - DNA, 17 bp, synthetic construct
  source 1..17: mol_type = other DNA
ccgtcaagctggagcct

SEQ ID NO: 30 - DNA, 18 bp, synthetic construct
  source 1..18: mol_type = other DNA
accgtcaagctggagcct

SEQ ID NO: 31 - DNA, 19 bp, synthetic construct
  source 1..19: mol_type = other DNA
taccgtcaagctggagcct

SEQ ID NO: 32 - DNA, 21 bp, synthetic construct
  source 1..21: mol_type = other DNA
aataccgtcaagctggagcct

SEQ ID NO: 33 - DNA, 22 bp, synthetic construct
  source 1..22: mol_type = other DNA
aaataccgtcaagctggagcct

SEQ ID NO: 34 - DNA, 23 bp, synthetic construct
  source 1..23: mol_type = other DNA
caaataccgtcaagctggagcct

SEQ ID NO: 35 - DNA, 24 bp, synthetic construct
  source 1..24: mol_type = other DNA
ccaaataccgtcaagctggagcct

SEQ ID NO: 36 - DNA, 25 bp, synthetic construct
  source 1..25: mol_type = other DNA
tccaaataccgtcaagctggagcct

SEQ ID NO: 37 - DNA, 20 bp, synthetic construct
  source 1..20: mol_type = other DNA
cgtcaagctggagcctcggt

SEQ ID NO: 38 - DNA, 15 bp, synthetic construct
  source 1..15: mol_type = other DNA
agctggagcctcggt

SEQ ID NO: 39 - DNA, 16 bp, synthetic construct
  source 1..16: mol_type = other DNA
aagctggagcctcggt

SEQ ID NO: 40 - DNA, 17 bp, synthetic construct
  source 1..17: mol_type = other DNA
caagctggagcctcggt

SEQ ID NO: 41 - DNA, 18 bp, synthetic construct
  source 1..18: mol_type = other DNA
tcaagctggagcctcggt

SEQ ID NO: 42 - DNA, 19 bp, synthetic construct
  source 1..19: mol_type = other DNA
gtcaagctggagcctcggt

SEQ ID NO: 43 - DNA, 21 bp, synthetic construct
  source 1..21: mol_type = other DNA
ccgtcaagctggagcctcggt

SEQ ID NO: 44 - DNA, 22 bp, synthetic construct
  source 1..22: mol_type = other DNA
accgtcaagctggagcctcggt

SEQ ID NO: 45 - DNA, 23 bp, synthetic construct
  source 1..23: mol_type = other DNA
taccgtcaagctggagcctcggt

SEQ ID NO: 46 - DNA, 24 bp, synthetic construct
  source 1..24: mol_type = other DNA
ataccgtcaagctggagcctcggt

SEQ ID NO: 47 - DNA, 25 bp, synthetic construct
  source 1..25: mol_type = other DNA
aataccgtcaagctggagcctcggt

SEQ ID NO: 48 - DNA, 20 bp, synthetic construct
  source 1..20: mol_type = other DNA
taccgtcaagctggagcctc

SEQ ID NO: 49 - DNA, 15 bp, synthetic construct
  source 1..15: mol_type = other DNA
tcaagctggagcctc

SEQ ID NO: 50 - DNA, 16 bp, synthetic construct
  source 1..16: mol_type = other DNA
gtcaagctggagcctc

SEQ ID NO: 51 - DNA, 17 bp, synthetic construct
  source 1..17: mol_type = other DNA
cgtcaagctggagcctc

SEQ ID NO: 52 - DNA, 18 bp, synthetic construct
  source 1..18: mol_type = other DNA
ccgtcaagctggagcctc

SEQ ID NO: 53 - DNA, 19 bp, synthetic construct
  source 1..19: mol_type = other DNA
accgtcaagctggagcctc

SEQ ID NO: 54 - DNA, 21 bp, synthetic construct
  source 1..21: mol_type = other DNA
ataccgtcaagctggagcctc

SEQ ID NO: 55 - DNA, 22 bp, synthetic construct
  source 1..22: mol_type = other DNA
aataccgtcaagctggagcctc

SEQ ID NO: 56 - DNA, 23 bp, synthetic construct
  source 1..23: mol_type = other DNA
aaataccgtcaagctggagcctc

SEQ ID NO: 57 - DNA, 24 bp, synthetic construct
  source 1..24: mol_type = other DNA
caaataccgtcaagctggagcctc

SEQ ID NO: 58 - DNA, 25 bp, synthetic construct
  source 1..25: mol_type = other DNA
ccaaataccgtcaagctggagcctc

SEQ ID NO: 59 - DNA, 20 bp, synthetic construct
  source 1..20: mol_type = other DNA
aataccgtcaagctggagcc

SEQ ID NO: 60 - DNA, 16 bp, synthetic construct
  source 1..16: mol_type = other DNA
ccgtcaagctggagcc

SEQ ID NO: 61 - DNA, 20 bp, synthetic construct
  source 1..20: mol_type = other DNA
gtcaagctggagcctcggta

SEQ ID NO: 62 - DNA, 16 bp, synthetic construct
  source 1..16: mol_type = other DNA
agctggagcctcggta

SEQ ID NO: 63 - DNA, 289 bp, synthetic construct
  source 1..289: mol_type = other DNA
ttctgtgagcaccgtgctgacctccaaataccgtcaagctggagcctcggtagccgttcctcctgcccgctgggcctcccaacgggccctcctcccctccttgcaccggcccttcctggtctttgaataaagtctgagtgggcagcagcctgtgtgtgcctgggttctctctatcccggaatgtgccaacaatggaggtgtttacctgtctcagaccaaggacctctctgcagctgcatggggctggggagggagaactgcagggagtatgggaggggaagctgaggtg

SEQ ID NO: 64 - DNA, 101 bp, synthetic construct
  source 1..101: mol_type = other DNA
ccgttgggaggcccagcgggcaggaggaacggctaccgaggctccagcttaacggtatttggaggtcagcacggtgctcacagaagccaggaacttgtcca

SEQ ID NO: 65 - RNA, 80 nt, synthetic construct
  source 1..80: mol_type = other RNA
gttttagagctagaaatagcaagttaaaataaggctagtccgttatcaacttgaaaaagtggcaccgagtcggtgctttt

SEQ ID NO: 66 - RNA, 100 nt, synthetic construct
  source 1..100: mol_type = other RNA
ccgtcaagctggagcctcgggttttagagctagaaatagcaagttaaaataaggctagtccgttatcaacttgaaaaagtggcaccgagtcggtgctttt

SEQ ID NO: 67 - RNA, 76 nt, synthetic construct
  source 1..76: mol_type = other RNA
gttttagagctagaaatagcaagttaaaataaggctagtccgttatcaacttgaaaaagtggcaccgagtcggtgc

SEQ ID NO: 68 - DNA, 24 bp, synthetic construct
  source 1..24: mol_type = other DNA
cgacaagcagaagaacggcatcaa

SEQ ID NO: 69 - DNA, 20 bp, synthetic construct
  source 1..20: mol_type = other DNA
cagctgcagagaggtccttg